European Patent Specification EP 3 837 274 B1, published November 6, 2024. Title: Acetyl-CoA Carboxylase2 Antisense Oligonucleotides. Applicant: OliPass Corporation Han, Seon-Young Sung, Kiho Hong, Myunghyo Kang, Dayoung Heo, Jeong-Seok Jang, Kang Won. The sequence listing filed with the application follows.

SEQUENCE LISTING (6 sequences)

SEQ ID NO: 1 - DNA, 14 bp, Artificial
  PNA modified oligonucleotide
  misc_feature (1)..(14): PNA modified oligonucleotide, human acetyl-CoA carboxylase2 targeted artificial sequence
  misc_feature (1)..(1): Carbamated N-terminal
  modified_base (3)..(3): n is a, g, c, or t
  modified_base (6)..(6): n is a, g, c, or t
  modified_base (8)..(8): n is a, g, c, or t
  modified_base (11)..(11): n is a, g, c, or t
  modified_base (13)..(13): n is a, g, c, or t
ctnacnanatngnc

SEQ ID NO: 2 - DNA, 16 bp, Artificial
  PNA modified oligonucleotide
  misc_feature (1)..(16): PNA modified oligonucleotide, human acetyl-CoA carboxylase2 targeted artificial sequence
  misc_feature (1)..(1): Carbamated N-terminal
  modified_base (2)..(3): n is a, g, c, or t
  modified_base (6)..(6): n is a, g, c, or t
  modified_base (9)..(9): n is a, g, c, or t
  modified_base (11)..(11): n is a, g, c, or t
  modified_base (13)..(13): n is a, g, c, or t
  modified_base (15)..(15): n is a, g, c, or t
tnntgncgnantngnc

SEQ ID NO: 3 - DNA, 14 bp, Artificial
  PNA modified oligonucleotide
  misc_feature (1)..(14): PNA modified oligonucleotide, human acetyl-CoA carboxylase2 targeted artificial sequence
  misc_feature (1)..(1): Carbamated N-terminal
  modified_base (2)..(2): n is a, g, c, or t
  modified_base (5)..(5): n is a, g, c, or t
  modified_base (7)..(7): n is a, g, c, or t
  modified_base (9)..(9): n is a, g, c, or t
  modified_base (11)..(11): n is a, g, c, or t
  modified_base (13)..(13): n is a, g, c, or t
tnctnangnantng

SEQ ID NO: 4 - DNA, 14 bp, Artificial
  PNA modified oligonucleotide
  misc_feature (1)..(14): PNA modified oligonucleotide, human acetyl-CoA carboxylase2 targeted artificial sequence
  misc_feature (1)..(1): Carbamated N-terminal
  modified_base (2)..(2): n is a, g, c, or t
  modified_base (5)..(5): n is a, g, c, or t
  modified_base (8)..(8): n is a, g, c, or t
  modified_base (10)..(10): n is a, g, c, or t
  modified_base (12)..(12): n is a, g, c, or t
  modified_base (14)..(14): n is a, g, c, or t
antgncgnantngn

SEQ ID NO: 5 - DNA, 12 bp, Artificial
  PNA modified oligonucleotide
  misc_feature (1)..(12): PNA modified oligonucleotide, human acetyl-CoA carboxylase2 targeted artificial sequence
  misc_feature (1)..(1): Carbamated N-terminal
  modified_base (3)..(3): n is a, g, c, or t
  modified_base (5)..(5): n is a, g, c, or t
  modified_base (7)..(7): n is a, g, c, or t
  modified_base (9)..(9): n is a, g, c, or t
  modified_base (11)..(11): n is a, g, c, or t
ctnangnantng

SEQ ID NO: 6 - DNA, 14 bp, Artificial
  PNA modified oligonucleotide
  misc_feature (1)..(14): PNA modified oligonucleotide, human acetyl-CoA carboxylase2 targeted artificial sequence
  misc_feature (1)..(1): Carbamated N-terminal
  modified_base (3)..(3): n is a, g, c, or t
  modified_base (5)..(5): n is a, g, c, or t
  modified_base (7)..(7): n is a, g, c, or t
  modified_base (9)..(9): n is a, g, c, or t
  modified_base (11)..(11): n is a, g, c, or t
  modified_base (13)..(13): n is a, g, c, or t
ctnangnantngnc